European Patent Application EP 4 570 834 A1, published June 18, 2025. Title: Affibody Micelle Drug Conjugate. Applicant: 興和株式会社. The sequence listing filed with the application follows.

SEQUENCE LISTING (11 sequences)

SEQ ID NO: 1 - protein, 58 aa, synthetic construct [sequence omitted]

SEQ ID NO: 2 - protein, 58 aa, synthetic construct
  source 1..58: note = Engineered HER2 binding polypeptide
AEAKYAKEMRNAYWEIALLPNLTNQQKRAFIRKLYDDPSQSSELLSEAKKLNDSQAPK

SEQ ID NO: 3 - protein, 58 aa, synthetic construct
  source 1..58: note = Engineered HER3 binding polypeptide
AEAKYAKEKYNAYYEIWQLPNLTKYQKAAFIGKLQDDPSQSSELLSEAKKLNDSQAPK

SEQ ID NO: 4 - protein, 58 aa, synthetic construct
  source 1..58: note = Engineered EGFR binding polypeptide
VDNKFNKEMWAAWEEIRNLPNLNGWQMTAFIASLVDDPSQSANLLAEAKKLNDAQAPK

SEQ ID NO: 5 - protein, 58 aa, synthetic construct
  source 1..58: note = Engineered EGFR binding polypeptide
VDNKFNKEMWIAWEEIRDLPNLNGWQMTAFIASLLDDPSQSANLLAEAKKLNDAQAPK

SEQ ID NO: 6 - protein, 58 aa, synthetic construct
  source 1..58: note = Engineered EGFR binding polypeptide
AEAKYAKEMWIAWEEIRNLPNLNGWQMTAFIAKLLDDPSQSSELLSEAKKLNDSQAPK

SEQ ID NO: 7 - protein, 58 aa, synthetic construct
  source 1..58: note = Engineered PD-L1 binding polypeptide
AEAKYAKERNAAAYEILYLPNLTNAQKWAFIWKLDDDPSQSSELLSEAKKLNDSQAPK

SEQ ID NO: 8 - protein, 58 aa, synthetic construct
  source 1..58: note = Engineered PD-L1 binding polypeptide
AEAKYAKERNKAAYEILYLPNLTNAQKWAFIWKLDDDPSQSSELLSEAKKLNDSQAPK

SEQ ID NO: 9 - protein, 68 aa, synthetic construct
  source 1..68: note = Engineered HER2 binding polypeptide
MHHHHHHAEAKYAKEMRNAYWEIALLPNLTNQQKRAFIRKLYDDPSQSSELLSEAKKLNDSQAPKVDC

SEQ ID NO: 10 - protein, 68 aa, synthetic construct
  source 1..68: note = Engineered EGFR binding polypeptide
MHHHHHHAEAKYAKEMWIAWEEIRNLPNLNGWQMTAFIAKLLDDPSQSSELLSEAKKLNDSQAPKVDC

SEQ ID NO: 11 - protein, 68 aa, synthetic construct
  source 1..68: note = Engineered HER3 binding polypeptide
MHEHEHEAEAKYAKEKYNAYYEIWQLPNLTKYQKAAFIGKLQDDPSQSSELLSEAKKLNDSQAPKVDC